European Patent Specification EP 3 999 512 B1, published August 23, 2023. Title: PYRAZOLO[3,4-d]PYRROLO[1,2-b]PYRIDAZINYL COMPOUNDS USEFUL AS IRAK4 INHIBITORS. Applicant: BRISTOL-MYERS SQUIBB COMPANY. The sequence listing filed with the application follows.

SEQUENCE LISTING (1 sequence)

SEQ ID NO: 1 - protein, 16 aa, Homo sapiens
  misc_feature: Flourescent tag attached to amino acid 1
IPTSPITTTYFFFKKK